European Patent Application EP 4 223 868 A1, published August 9, 2023. Title: Enhancement of Anti-tumor Effects of Immune Checkpoint Inhibitors by administering of Ruminococcaceae Intestinal Bacteria. Applicant: NATIONAL CANCER CENTER RIKEN. The sequence listing filed with the application follows.

SEQUENCE LISTING (1 sequence)

SEQ ID NO: 1 - DNA, 1478 bp, Ruminococcaceae unclassified genus
agagtttgatcctggctcaggacgaacgctggcggcgtgcctaacacatgcaagtcgaacggagttgaaaggagcttgcttttttcaacttagtggcggacgggtgagtaacgcgtgagtaacctgcctttcagagggggataacgttctgaaaagaacgctaataccgcataagattgtagcttcgcatggagcagcaatcaaaggagcaatccgctgaaagatggactcgcgtccgattagatagttggcggggtaacggcccaccaagtcgacgatcggtagccggactgagaggttgatcggccacattgggactgagacacggcccagactcctacgggaggcagcagtgagggatattgggcaatgggggaaaccctgacccagcaacgccgcgtgagggatgacggttttcggattgtaaacctctgtcctctgtgaagatagtgacggtagcagaggaggaagctccggctaactacgtgccagcagccgcggtaatacgtagggagcaagcgttgtccggatttactgggtgtaaagggtgcgtaggcggattggcaagtcagaagtgaaatccatgggcttaacccatgaactgcttttgaaactgttagtcttgagtgaagtagaggtaggcggaattcccggtgtagcggtgaaatgcgtagagatcgggaggaacaccagtggcgaaggcggcctactgggctttaactgacgctgaggcacgaaagtgtgggtagcaaacaggattagataccctggtagtccacactgtaaacgatgattactaggtgtggggggtctaaccccctccgtgccggagttaacacaataagtaatccacctggggagtacgaccgcaaggttgaaactcaaaggaattgacgggggcccgcacaagcagtggagtatgtggtttaattcgacgcaacgcgaagaaccttaccaggtcttgacatccaactaacgaagcagagatgcattaggtgcccttcggggaaagttgagacaggtggtgcatggttgtcgtcagctcgtgtcgtgagatgttgggttaagtcccgcaacgagcgcaacccttgtgattagttgctacgcaagagcactctaatcagactgccgttgacaaaacggaggaaggtggggacgacgtcaaatcatcatgccctttatgacctgggctacacacgtactacaatggtcgttaacagagggaagcaataccgcgaggtggagcaaaaccctaaaaacggtctcagttcagattgtaggctgcaactcgcctacatgaagttggaattgctagtaatcgcggatcagcatgccgcggtgaatacgttcccgggccttgtacacaccgcccgtcacaccatgggagccggtaatacccgaagtcagtagtttaaccgtaaggagaacgctgccgaaggtaggattggcgactggggtgaagtcgtaacaaggtaacc